European Patent Specification EP 3 956 455 B1, published July 26, 2023. Title: Method and kit for the identification of Vaccinium myrtillus. Applicant: INDENA S.p.A. The sequence listing filed with the application follows.

SEQUENCE LISTING (14 sequences)

SEQ ID NO: 1 - DNA, 131 bp, Unknown
  Vaccinium myrtillus
gcattgcgtcacccactccccccgtgccccaagcgggcacgtcggagcgtgggcggatattggccccccgttcgcatccgtgcgcggtcggcctaaaaaacgggtccccaatgacggacatcacgacaagt

SEQ ID NO: 2 - DNA, 170 bp, Unknown
  Vaccinium myrtillus
tgaaggcacgtctgcctgggcgtcacgcattgcgtcacccactccccccgtgccccaagcgggcacgtcggagcgtgggcggatattggccccccgttcgcatccgtgcgcggtcggcctaaaaaacgggtccccaatgacggacatcacgacaagtggtggttgctaaa

SEQ ID NO: 3 - DNA, 230 bp, Unknown
  Vaccinium myrtillus
ttgcagaatcccgtgaaccatcgagtctttgaacgcaagttgcgcctgaagccattaggttgaaggcacgtctgcctgggcgtcacgcattgcgtcacccactccccccgtgccccaagcgggcacgtcggagcgtgggcggatattggccccccgttcgcatccgtgcgcggtcggcctaaaaaacgggtccccaatgacggacatcacgacaagtggtggttgctaaa

SEQ ID NO: 4 - DNA, 275 bp, Unknown
  Vaccinium myrtillus
ccatcgagtctttgaacgcaagttgcgcctgaagccattaggttgaaggcacgtctgcctgggcgtcacgcattgcgtcacccactccccccgtgccccaagcgggcacgtcggagcgtgggcggatattggccccccgttcgcatccgtgcgcggtcggcctaaaaaacgggtccccaatgacggacatcacgacaagtggtggttgctaaaccgtcgcgtcacgtcgtgcatgccatcgtttgttgcgggttggcccatttgaccctgaagtg

SEQ ID NO: 5 - DNA, 18 bp, Artificial Sequence
  oligonucleotide primer
gcattgcgtcacccactc

SEQ ID NO: 6 - DNA, 22 bp, Artificial Sequence
  oligonucleotide primer
acttgtcgttgaatgtccgtca

SEQ ID NO: 7 - DNA, 18 bp, Artificial Sequence
  oligonucleotide primer
tgaaggcacgtctgcctg

SEQ ID NO: 8 - DNA, 22 bp, Artificial Sequence
  oligonucleotide primer
tttagcaaccaccacttgtcgt

SEQ ID NO: 9 - DNA, 20 bp, Artificial Sequence
  oligonucleotide primer
ttgcagaatcccgtgaacca

SEQ ID NO: 10 - DNA, 22 bp, Artificial Sequence
  oligonucleotide primer
tttagcaaccaccacttgtcgt

SEQ ID NO: 11 - DNA, 20 bp, Artificial Sequence
  oligonucleotide primer
ccatcgagtctttgaacgca

SEQ ID NO: 12 - DNA, 20 bp, Artificial Sequence
  oligonucleotide primer
cacttcagggtcaaatgggc

SEQ ID NO: 13 - DNA, 16 bp, Artificial Sequence
  oligonucleotide probe
acgtcggagcgtgggc

SEQ ID NO: 14 - DNA, 18 bp, Artificial Sequence
  oligonucleotide probe
tagggcgggtaagtgagt